European Patent Application EP 4 717 776 A2, published April 1, 2026. Title: POLYPEPTIDE CONJUGATES FOR INTRACELLULAR DELIVERY OF NUCLEIC ACIDS. Applicant: OHIO STATE INNOVATION FOUNDATION. The sequence listing filed with the application follows.

SEQUENCE LISTING (145 sequences)

SEQ ID NO: 1 - protein, 6 aa, synthetic construct
  REGION 1..6: note = synthetic construct
  SITE 2: note = X is L-2-naphthylalanine
FARRRQ

SEQ ID NO: 2 - protein, 6 aa, synthetic construct
  REGION 1..6: note = synthetic construct
  SITE 2: note = X is L-2-naphthylalanine
FARRRC

SEQ ID NO: 3 - protein, 6 aa, synthetic construct
  REGION 1..6: note = synthetic construct
  SITE 2: note = X is L-2-naphthylalanine
FARRRO

SEQ ID NO: 4 - protein, 6 aa, synthetic construct
  REGION 1..6: note = synthetic construct
  SITE 4: note = X is L-2-naphthylalanine
RRRAFQ

SEQ ID NO: 5 - protein, 6 aa, synthetic construct
  REGION 1..6: note = synthetic construct
  SITE 5: note = X is L-2-naphthylalanine
RRRRAF

SEQ ID NO: 6 - protein, 6 aa, synthetic construct
  REGION 1..6: note = synthetic construct
  SITE 2: note = X is L-2-naphthylalanine
FARRRR

SEQ ID NO: 7 - protein, 7 aa, synthetic construct
  REGION 1..7: note = synthetic construct
  SITE 2: note = X is D-2-naphthylalanine
  SITE 3: note = X is D-arginine
  SITE 5: note = X is D-arginine
  SITE 7: note = X is D-glutamine
FARRRRQ

SEQ ID NO: 8 - protein, 7 aa, synthetic construct
  REGION 1..7: note = synthetic construct
  SITE 2: note = X is D-2-naphthylalanine
  SITE 3: note = X is D-arginine
  SITE 5: note = X is D-arginine
FARRRRQ

SEQ ID NO: 9 - protein, 7 aa, synthetic construct
  REGION 1..7: note = synthetic construct
  SITE 2: note = X is L-2-naphthylalanine
FARRRRQ

SEQ ID NO: 10 - protein, 7 aa, synthetic construct
  REGION 1..7: note = synthetic construct
  SITE 1: note = X is D-phenylalanine
  SITE 2: note = X is L-2-naphthylalanine
  SITE 4: note = X is D-arginine
  SITE 6: note = X is D-arginine
FARRRRQ

SEQ ID NO: 11 - protein, 7 aa, synthetic construct
  REGION 1..7: note = synthetic construct
  SITE 5: note = X is L-2-naphthylalanine
RRFRARQ

SEQ ID NO: 12 - protein, 7 aa, synthetic construct
  REGION 1..7: note = synthetic construct
  SITE 6: note = X is L-2-naphthylalanine
FRRRRAQ

SEQ ID NO: 13 - protein, 7 aa, synthetic construct
  REGION 1..7: note = synthetic construct
  SITE 1: note = X is D-arginine
  SITE 5: note = X is L-2-naphthylalanine
RRFRARQ

SEQ ID NO: 14 - protein, 7 aa, synthetic construct
  REGION 1..7: note = synthetic construct
  SITE 3: note = X is L-2-naphthylalanine
RRAFRRQ

SEQ ID NO: 15 - protein, 8 aa, synthetic construct
  REGION 1..8: note = synthetic construct
CRRRRFWQ

SEQ ID NO: 16 - protein, 8 aa, synthetic construct
  REGION 1..8: note = synthetic construct
  SITE 2: note = X is D-phenylalanine
  SITE 3: note = X is L-2-naphthylalanine
  SITE 5: note = X is D-arginine
  SITE 7: note = X is D-arginine
FFARRRRQ

SEQ ID NO: 17 - protein, 8 aa, synthetic construct
  REGION 1..8: note = synthetic construct
  SITE 3: note = X is L-2-naphthylalanine
FFARRRRQ

SEQ ID NO: 18 - protein, 8 aa, synthetic construct
  REGION 1..8: note = synthetic construct
  SITE 6: note = X is L-2-naphthylalanine
RFRFRARQ

SEQ ID NO: 19 - protein, 8 aa, synthetic construct
  REGION 1..8: note = synthetic construct
ORRRRFWQ

SEQ ID NO: 20 - protein, 8 aa, synthetic construct
  REGION 1..8: note = synthetic construct
CRRRRFWQ

SEQ ID NO: 21 - protein, 8 aa, synthetic construct
  REGION 1..8: note = synthetic construct
  SITE 2: note = X is L-2-naphthylalanine
FARRRRQK

SEQ ID NO: 22 - protein, 8 aa, synthetic construct
  REGION 1..8: note = synthetic construct
  SITE 2: note = X is L-2-naphthylalanine
FARRRRQC

SEQ ID NO: 23 - protein, 8 aa, synthetic construct
  REGION 1..8: note = synthetic construct
  SITE 1: note = X is D-phenylalanine
  SITE 2: note = X is L-2-naphthylalanine
  SITE 4: note = X is D-arginine
  SITE 6: note = X is D-arginine
FARRRRRQ

SEQ ID NO: 24 - protein, 8 aa, synthetic construct
  REGION 1..8: note = synthetic construct
  SITE 2: note = X is L-2-naphthylalanine
FARRRRRQ

SEQ ID NO: 25 - protein, 9 aa, synthetic construct
  REGION 1..9: note = synthetic construct
  SITE 5: note = X is L-2-naphthylalanine
  SITE 8: note = X is L-Nle
RRRRAFDXC

SEQ ID NO: 26 - protein, 5 aa, synthetic construct
  REGION 1..5: note = synthetic construct
  SITE 2: note = X is L-2-naphthylalanine
FARRR

SEQ ID NO: 27 - protein, 5 aa, synthetic construct
  REGION 1..5: note = synthetic construct
FWRRR

SEQ ID NO: 28 - protein, 5 aa, synthetic construct
  REGION 1..5: note = synthetic construct
  SITE 4: note = X is L-2-naphthylalanine
RRRAF

SEQ ID NO: 29 - protein, 5 aa, synthetic construct
  REGION 1..5: note = synthetic construct
RRRWF

SEQ ID NO: 30 - protein, 7 aa, synthetic construct
  REGION 1..7: note = synthetic construct
  SITE 2: note = X is L-2-naphthylalanine
FARRRRQ

SEQ ID NO: 31 - protein, 6 aa, synthetic construct
  REGION 1..6: note = synthetic construct
FFRRRQ

SEQ ID NO: 32 - protein, 6 aa, synthetic construct
  REGION 1..6: note = synthetic construct
  SITE 3: note = X is D-arginine
  SITE 5: note = X is D-arginine
FFRRRQ

SEQ ID NO: 33 - protein, 6 aa, synthetic construct
  REGION 1..6: note = synthetic construct
  SITE 4: note = X is D-arginine
FFRRRQ

SEQ ID NO: 34 - protein, 6 aa, synthetic construct
  REGION 1..6: note = synthetic construct
FRFRRQ

SEQ ID NO: 35 - protein, 6 aa, synthetic construct
  REGION 1..6: note = synthetic construct
FRRFRQ

SEQ ID NO: 36 - protein, 6 aa, synthetic construct
  REGION 1..6: note = synthetic construct
FRRRFQ

SEQ ID NO: 37 - protein, 6 aa, synthetic construct
  REGION 1..6: note = synthetic construct
  SITE 2: note = X is L-2-naphthylalanine
GARRRQ

SEQ ID NO: 38 - protein, 6 aa, synthetic construct
  REGION 1..6: note = synthetic construct
FFFRAQ

SEQ ID NO: 39 - protein, 6 aa, synthetic construct
  REGION 1..6: note = synthetic construct
FFFRRQ

SEQ ID NO: 40 - protein, 7 aa, synthetic construct
  REGION 1..7: note = synthetic construct
FFRRRRQ

SEQ ID NO: 41 - protein, 7 aa, synthetic construct
  REGION 1..7: note = synthetic construct
FRRFRRQ

SEQ ID NO: 42 - protein, 7 aa, synthetic construct
  REGION 1..7: note = synthetic construct
FRRRFRQ

SEQ ID NO: 43 - protein, 7 aa, synthetic construct
  REGION 1..7: note = synthetic construct
RFFRRRQ

SEQ ID NO: 44 - protein, 7 aa, synthetic construct
  REGION 1..7: note = synthetic construct
RFRRFRQ

SEQ ID NO: 45 - protein, 7 aa, synthetic construct
  REGION 1..7: note = synthetic construct
FRFRRRQ

SEQ ID NO: 46 - protein, 7 aa, synthetic construct
  REGION 1..7: note = synthetic construct
FFFRRRQ

SEQ ID NO: 47 - protein, 6 aa, synthetic construct
  REGION 1..6: note = synthetic construct
FFRRRF

SEQ ID NO: 48 - protein, 7 aa, synthetic construct
  REGION 1..7: note = synthetic construct
FRFFRRQ

SEQ ID NO: 49 - protein, 7 aa, synthetic construct
  REGION 1..7: note = synthetic construct
RRFFFRQ

SEQ ID NO: 50 - protein, 7 aa, synthetic construct
  REGION 1..7: note = synthetic construct
FFRFRRQ

SEQ ID NO: 51 - protein, 7 aa, synthetic construct
  REGION 1..7: note = synthetic construct
FFRRFRQ

SEQ ID NO: 52 - protein, 7 aa, synthetic construct
  REGION 1..7: note = synthetic construct
FRRFFRQ

SEQ ID NO: 53 - protein, 7 aa, synthetic construct
  REGION 1..7: note = synthetic construct
FRRFRFQ

SEQ ID NO: 54 - protein, 7 aa, synthetic construct
  REGION 1..7: note = synthetic construct
FRFRFRQ

SEQ ID NO: 55 - protein, 7 aa, synthetic construct
  REGION 1..7: note = synthetic construct
RFFRFRQ

SEQ ID NO: 56 - protein, 7 aa, synthetic construct
  REGION 1..7: note = synthetic construct
  SITE 2: note = X is L-2-naphthylalanine
GARRRRQ

SEQ ID NO: 57 - protein, 8 aa, synthetic construct
  REGION 1..8: note = synthetic construct
FFFRRRRQ

SEQ ID NO: 58 - protein, 8 aa, synthetic construct
  REGION 1..8: note = synthetic construct
RFFRRRRQ

SEQ ID NO: 59 - protein, 7 aa, synthetic construct
  REGION 1..7: note = synthetic construct
RRFFRRR

SEQ ID NO: 60 - protein, 8 aa, synthetic construct
  REGION 1..8: note = synthetic construct
RFFFRRRQ

SEQ ID NO: 61 - protein, 8 aa, synthetic construct
  REGION 1..8: note = synthetic construct
RRFFFRRQ

SEQ ID NO: 62 - protein, 8 aa, synthetic construct
  REGION 1..8: note = synthetic construct
FFRRFRRQ

SEQ ID NO: 63 - protein, 8 aa, synthetic construct
  REGION 1..8: note = synthetic construct
FFRRRRFQ

SEQ ID NO: 64 - protein, 8 aa, synthetic construct
  REGION 1..8: note = synthetic construct
FRRFFRRQ

SEQ ID NO: 65 - protein, 9 aa, synthetic construct
  REGION 1..9: note = synthetic construct
FFFRRRRRQ

SEQ ID NO: 66 - protein, 10 aa, synthetic construct
  REGION 1..10: note = synthetic construct
FFFRRRRRRQ

SEQ ID NO: 67 - protein, 7 aa, synthetic construct
  REGION 1..7: note = synthetic construct
  SITE 2: note = X is L-2-naphthylalanine
  SITE 4: note = X is D-arginine
  SITE 6: note = X is D-arginine
FARRRRQ

SEQ ID NO: 68 - protein, 7 aa, synthetic construct
  REGION 1..7: note = synthetic construct
  VARIANT 1..2: note = X can be any naturally occurring amino acid
XXRRRRQ

SEQ ID NO: 69 - protein, 7 aa, synthetic construct
  REGION 1..7: note = synthetic construct
  SITE 2: note = X is D-phenylalanine
  SITE 5: note = X is D-arginine
FFFRRRQ

SEQ ID NO: 70 - protein, 7 aa, synthetic construct
  REGION 1..7: note = synthetic construct
  SITE 1: note = X is D-phenylalanine
  SITE 3: note = X is D-phenylalanine
  SITE 4: note = X is D-arginine
  SITE 6: note = X is D-arginine
FFFRRRQ

SEQ ID NO: 71 - protein, 7 aa, synthetic construct
  REGION 1..7: note = synthetic construct
  SITE 1: note = X is D-phenylalanine
  SITE 3: note = X is D-phenylalanine
  SITE 5: note = X is D-arginine
FFFRRRQ

SEQ ID NO: 72 - protein, 7 aa, synthetic construct
  REGION 1..7: note = synthetic construct
  SITE 2: note = X is D-phenylalanine
  SITE 4: note = X is D-arginine
  SITE 6: note = X is D-arginine
FFFRRRQ

SEQ ID NO: 73 - protein, 7 aa, synthetic construct
  REGION 1..7: note = synthetic construct
  SITE 1: note = X is D-phenylalanine
  SITE 3: note = X is L-2-naphthylalanine
  SITE 4: note = X is D-arginine
  SITE 6: note = X is D-arginine
FFARRRQ

SEQ ID NO: 74 - protein, 7 aa, synthetic construct
  REGION 1..7: note = synthetic construct
  SITE 1: note = X is D-phenylalanine
  SITE 2: note = X is L-2-naphthylalanine
  SITE 3: note = X is D-phenylalanine
  SITE 4: note = X is D-arginine
  SITE 6: note = X is D-arginine
FAFRRRQ

SEQ ID NO: 75 - protein, 7 aa, synthetic construct
  REGION 1..7: note = synthetic construct
  SITE 1: note = X is L-2-naphthylalanine
  SITE 3: note = X is D-phenylalanine
  SITE 4: note = X is D-arginine
  SITE 6: note = X is D-arginine
AFFRRRQ

SEQ ID NO: 76 - protein, 6 aa, synthetic construct
  REGION 1..6: note = synthetic construct
  SITE 2: note = X is L-2-naphthylalanine
  SITE 3: note = X is D-arginine
  SITE 5: note = X is D-arginine
FARRRQ

SEQ ID NO: 77 - protein, 6 aa, synthetic construct
  REGION 1..6: note = synthetic construct
  SITE 1: note = X is D-phenylalanine
  SITE 2: note = X is L-2-naphthylalanine
  SITE 3: note = X is D-arginine
  SITE 5: note = X is D-arginine
FARRRQ

SEQ ID NO: 78 - protein, 8 aa, synthetic construct
  REGION 1..8: note = synthetic construct
  MOD_RES 1: note = ACETYLATION
  SITE 2: note = X is D-phenylalanine
  SITE 5: note = X is D-arginine
  SITE 7: note = X is D-arginine
KFFRRRRD

SEQ ID NO: 79 - protein, 8 aa, synthetic construct
  REGION 1..8: note = synthetic construct
  MOD_RES 1: note = ACETYLATION
  SITE 1: note = X is L-2,3-diaminopropionic acid
  SITE 2: note = X is D-phenylalanine
  SITE 5: note = X is D-arginine
  SITE 7: note = X is D-arginine
XRFRRRRD

SEQ ID NO: 80 - protein, 8 aa, synthetic construct
  REGION 1..8: note = synthetic construct
  DISULFID 1..8: note = Cys residues joined by disulfide bond
CWWRRRRC

SEQ ID NO: 81 - protein, 9 aa, synthetic construct
  REGION 1..9: note = synthetic construct
  DISULFID 1..9: note = Cys residues jopined by disulfide bond
CWWVRRRRC

SEQ ID NO: 82 - protein, 8 aa, synthetic construct
  REGION 1..8: note = synthetic construct
  DISULFID 1..8: note = Cys residues jopined by disulfide bond
CFWRRRRC

SEQ ID NO: 83 - protein, 8 aa, synthetic construct
  REGION 1..8: note = synthetic construct
  DISULFID 1..8: note = Cys residues jopined by disulfide bond
CWWWRRRC

SEQ ID NO: 84 - protein, 7 aa, synthetic construct
  REGION 1..7: note = synthetic construct
  SITE 1: note = X is L-homeoproline
  SITE 2: note = X is L-napthylalanine
  SITE 5: note = X is D-arginine
  SITE 6: note = X is D-arginine
  SITE 7: note = X is D-glutamate
PARERRE

SEQ ID NO: 85 - protein, 7 aa, synthetic construct
  REGION 1..7: note = synthetic construct
  SITE 1: note = X is L-homeoproline
  SITE 2: note = X is L-napthylalanine
  SITE 5: note = X is D-arginine
  SITE 6: note = X is D-arginine
  SITE 7: note = X is D-glutamate
PARRRRE

SEQ ID NO: 86 - protein, 7 aa, synthetic construct
  REGION 1..7: note = synthetic construct
  SITE 1: note = X is L-homeoproline
  SITE 2: note = X is L-napthylalanine
  SITE 2..3: note = X is L-napthylalanine
  SITE 5: note = X is D-arginine
  SITE 6: note = X is D-arginine
  SITE 7: note = X is D-glutamate
PAARRRE

SEQ ID NO: 87 - protein, 7 aa, synthetic construct
  REGION 1..7: note = synthetic construct
  SITE 1: note = X is L-homeoproline
  SITE 2: note = X is L-napthylalanine
  SITE 3: note = X is L-napthylalanine
  SITE 5: note = X is D-arginine
  SITE 6: note = X is D-arginine
PAARRRE

SEQ ID NO: 88 - protein, 7 aa, synthetic construct
  REGION 1..7: note = synthetic construct
  SITE 1: note = X is L-homeoproline
  SITE 2: note = X is L-napthylalanine
  SITE 5: note = X is D-arginine
  SITE 6: note = X is D-arginine
  SITE 7: note = X is D-glutamate
PAFRRRE

SEQ ID NO: 89 - protein, 7 aa, synthetic construct
  REGION 1..7: note = synthetic construct
  SITE 1: note = X is L-homeoproline
  SITE 2: note = X is L-napthylalanine
  SITE 5: note = X is D-arginine
  SITE 6: note = X is D-arginine
PAFRRRE

SEQ ID NO: 90 - protein, 7 aa, synthetic construct
  REGION 1..7: note = synthetic construct
  SITE 1: note = X is L-homeoproline
  SITE 2: note = X is L-napthylalanine
  SITE 3: note = X is D-phenylalanine
  SITE 5: note = X is D-arginine
  SITE 6: note = X is D-arginine
  SITE 7: note = X is D-glutamate
PAARRRE

SEQ ID NO: 91 - protein, 7 aa, synthetic construct
  REGION 1..7: note = synthetic construct
  SITE 1: note = X is L-homeoproline
  SITE 2: note = X is L-napthylalanine
  SITE 3: note = X is D-phenylalanine
  SITE 5: note = X is D-arginine
  SITE 6: note = X is D-arginine
PAARRRE

SEQ ID NO: 92 - protein, 7 aa, synthetic construct
  REGION 1..7: note = synthetic construct
  SITE 1: note = X is L-homeoproline
  SITE 2: note = X is L-napthylalanine
  SITE 3: note = X is D-napthylalanine
  SITE 5: note = X is D-arginine
  SITE 6: note = X is D-arginine
PAARRRE

SEQ ID NO: 93 - protein, 7 aa, synthetic construct
  REGION 1..7: note = synthetic construct
  SITE 1: note = X is L-homeoproline
  SITE 2: note = X is L-napthylalanine
  SITE 3: note = X is D-napthylalanine
  SITE 5: note = X is D-arginine
  SITE 6: note = X is D-arginine
  SITE 7: note = X is D-glutamate
PAARRRE

SEQ ID NO: 94 - protein, 8 aa, synthetic construct
  REGION 1..8: note = synthetic construct
  MOD_RES 1: note = Arg is modified with pimelic acid
  SITE 1..4: note = Cyclization between Arginine-Arginine amino acids
  SITE 4: note = Arg is modified with lysine peptoid residue
RQRRGRRR

SEQ ID NO: 95 - protein, 19 aa, synthetic construct
  REGION 1..19: note = synthetic construct
  DISULFID 2..19: note = Cys residues joined by disulfide bond
KCFQWQRNMRKVRGPPVSC

SEQ ID NO: 96 - protein, 11 aa, synthetic construct
  REGION 1..11: note = synthetic construct
  SITE 1..11: note = Cyclization between lysine and glutamic acid
  SITE 2: note = X is D-arginine
  SITE 4: note = X is D-arginine
  SITE 6: note = X is D-arginine
  SITE 8: note = X is D-lysine
  SITE 10: note = X is D-arginine
KRRRGRKKRRE

SEQ ID NO: 97 - protein, 12 aa, synthetic construct
  REGION 1..12: note = synthetic construct
  SITE 1..12: note = Cyclization between lysine and glutamic acid
  SITE 2: note = X is D-arginine
  SITE 4: note = X is D-arginine
  SITE 6: note = X is D-arginine
  SITE 8: note = X is D-arginine
  SITE 10: note = X is D-arginine
KRRRRRRRRRRE

SEQ ID NO: 98 - protein, 14 aa, synthetic construct
  REGION 1..14: note = synthetic construct
  SITE 13: note = X is D-proline
RVRTRGKRRIRRPP

SEQ ID NO: 99 - protein, 14 aa, synthetic construct
  REGION 1..14: note = synthetic construct
  SITE 13: note = X is D-proline
RTRTRGKRRIRVPP

SEQ ID NO: 100 - protein, 8 aa, synthetic construct
  REGION 1..8: note = synthetic construct
WRWRWRWR

SEQ ID NO: 101 - protein, 34 aa, synthetic construct
  REGION 1..34: note = synthetic construct
  DISULFID 4..21: note = Cys residues jopined by disulfide bond
  DISULFID 11..23: note = Cys residues jopined by disulfide bond
  DISULFID 17..29: note = Cys residues jopined by disulfide bond
GGVCPKILKKCRRDSDCPGACICRGNGYCGSGSD

SEQ ID NO: 102 - protein, 10 aa, synthetic construct
  REGION 1..10: note = synthetic construct
  MOD_RES 1..10: note = Macrocyclization by multicomponent reaction with aziridine aldehyde and isocyanide
  SITE 1..10: note = Macrocyclization between proline and lysine
  SITE 2: note = X is L-3-cyclohexyl-alanine
  SITE 3: note = X is D-arginine
  SITE 4: note = X is L-3-cyclohexyl-alanine
  SITE 5: note = X is D-arginine
  SITE 6: note = X is L-3-cyclohexyl-alanine
  SITE 7: note = X is D-arginine
  SITE 8: note = X is L-3-cyclohexyl-alanine
  SITE 9: note = X is D-arginine
PXRXRXRXRG

SEQ ID NO: 103 - protein, 13 aa, synthetic construct
  REGION 1..13: note = synthetic construct
  MOD_RES 1: note = Ser is modified with trimesic acid
  SITE 1..13: note = N-terminal amine and side chains of two L-2,3-diaminopropionic acid residues bicyclized with trimesic acid
  SITE 1..13: note = bicyclic bond between N-terminal serine and L-2,3-diaminopropionic acid
  SITE 2: note = X is D-valine
  SITE 4: note = X is L-difluorophosphonomethyl phenylalanine
  SITE 6: note = X is L-2,3-diaminopropionic acid
  SITE 8: note = X is L-2-naphthylalanine
  SITE 13: note = X is L-2,3-diaminopropionic acid
SVPXHXFARRRRX

SEQ ID NO: 104 - protein, 16 aa, synthetic construct
  REGION 1..16: note = synthetic construct
  SITE 1: note = D-alanine is modified with trimesic acid
  SITE 1: note = X is D-alanine
  SITE 1..16: note = N-terminal amine and side chains of two L-2,3-diaminopropionic acid residues bicyclized with trimesic acid
  SITE 1..16: note = bicyclic bond between N-terminal serine and L-2,3-diaminopropionic acid
  SITE 2: note = MeGly
  SITE 3: note = X is D-phosphothreonine
  SITE 4: note = X is L-piperidine-2-carboxylic acid
  SITE 5: note = X is L-2-naphthylalanine
  SITE 8: note = X is D-alanine
  SITE 9: note = X is L-2,3-diaminopropionic acid
  SITE 11: note = X is L-2-naphthylalanine
  SITE 16: note = X is L-2,3-diaminopropionic acid
AGTXARAAXFARRRRX

SEQ ID NO: 105 - protein, 16 aa, synthetic construct
  REGION 1..16: note = synthetic construct
  SITE 1..15: note = Three Cysinine side chains bicyclized with tris(bromomethyl)benzene
  SITE 1..9: note = Cysinine-Cysinine cyclic bone
  SITE 9..15: note = Cysinine-Cysinine cyclic bone
  SITE 1..15: note = Cysinine-Cysinine cyclic bone
CRRSRRGCGRRSRRCG

SEQ ID NO: 106 - protein, 5 aa, synthetic construct
  REGION 1..5: note = synthetic construct
  SITE 1..2: note = linked by dodecanoyl moiety
KRRRR

SEQ ID NO: 107 - protein, 16 aa, synthetic construct
  REGION 1..16: note = synthetic construct
LKKLCKLLKKLCKLAG

SEQ ID NO: 108 - protein, 9 aa, synthetic construct
  REGION 1..9: note = synthetic construct
  SITE 5..9: note = Cyclization between lysine and glutamic acid
RRRRKRRRE

SEQ ID NO: 109 - protein, 9 aa, synthetic construct
  REGION 1..9: note = synthetic construct
  SITE 4..9: note = Cyclization between lysine and Glutamic acid
RRRKRRRRE

SEQ ID NO: 110 - protein, 9 aa, synthetic construct
  REGION 1..9: note = synthetic construct
  SITE 3..9: note = Cyclization between lysine and Glutamic acid
RRKRRRRRE

SEQ ID NO: 111 - protein, 9 aa, synthetic construct
  REGION 1..9: note = synthetic construct
  SITE 2..9: note = Cyclization between lysine and Glutamic acid
RKRRRRRRE

SEQ ID NO: 112 - protein, 8 aa, synthetic construct
  REGION 1..8: note = synthetic construct
CRCRCRCR

SEQ ID NO: 113 - protein, 12 aa, synthetic construct
  REGION 1..12: note = synthetic construct
  SITE 1: note = X is L-propargylglycine
  SITE 1..12: note = Cyclization by the click reaction between L-propargylglycine and L-6-Azido-2-amino-hexanoic
  SITE 1..12: note = Cyclic bond between L-propargylglycine and L-6-Azido-2-amino-hexanoic
  SITE 12: note = X is L-6-Azido-2-amino-hexanoic
XLRKRLRKFRNX

SEQ ID NO: 114 - protein, 9 aa, synthetic construct
  REGION 1..9: note = synthetic construct
  SITE 2: note = X is L-2,3-diaminopropionic acid
  SITE 3: note = X is L-2,3-diaminopropionic acid
  SITE 4: note = X is L-2,3-diaminopropionic acid
  SITE 5: note = X is D-phenylalanine
  SITE 7: note = X is L-2,3-diaminopropionic acid
  SITE 8: note = X is L-2,3-diaminopropionic acid
TXXXFLXXT

SEQ ID NO: 115 - protein, 9 aa, synthetic construct
  REGION 1..9: note = synthetic construct
  SITE 2: note = X is L-2-amino-3-guanidinylpropionic acid
  SITE 3: note = X is L-2,3-diaminopropionic acid
  SITE 4: note = X is L-2-amino-3-guanidinylpropionic acid
  SITE 5: note = X is D-phenylalanine
  SITE 7: note = X is L-2-amino-3-guanidinylpropionic acid
  SITE 8: note = X is L-2-amino-3-guanidinylpropionic acid
TXXXFLXXT

SEQ ID NO: 116 - protein, 7 aa, synthetic construct
  REGION 1..7: note = synthetic construct
  SITE 2: note = X is L-2-naphthylalanine
FARRRRQ

SEQ ID NO: 117 - protein, 8 aa, synthetic construct
  REGION 1..8: note = synthetic construct
  SITE 2: note = X is D-phenylalanine
  SITE 3: note = X is L-2-naphthylalanine
  SITE 5: note = X is D-arginine
  SITE 7: note = X is D-arginine
FFARRRRQ

SEQ ID NO: 118 - protein, 7 aa, synthetic construct
  REGION 1..7: note = synthetic construct
  SITE 1: note = X is D-phenylalanine
  SITE 2: note = X is L-2-naphthylalanine
  SITE 4: note = X is D-arginine
  SITE 6: note = X is D-arginine
FARRRRQ

SEQ ID NO: 119 - protein, 8 aa, synthetic construct
  REGION 1..8: note = synthetic construct
  SITE 1: note = X is D-phenylalanine
  SITE 2: note = X is L-2-naphthylalanine
  SITE 4: note = X is D-arginine
  SITE 6: note = X is D-arginine
FARRRRRQ

SEQ ID NO: 120 - protein, 7 aa, synthetic construct
  REGION 1..7: note = synthetic construct
  SITE 2: note = X is D-2-naphthylalanine
  SITE 3: note = X is D-arginine
  SITE 5: note = X is D-arginine
  SITE 7: note = X is D-glutamine
FARRRRE

SEQ ID NO: 121 - protein, 7 aa, synthetic construct
  REGION 1..7: note = synthetic construct
  SITE 2: note = X is D-2-naphthylalanine
  SITE 3: note = X is D-arginine
  SITE 5: note = X is D-arginine
FARRRRQ

SEQ ID NO: 122 - protein, 8 aa, synthetic construct
  REGION 1..8: note = synthetic construct
  SITE 2: note = X is L-2-naphthylalanine
FARRRRRQ

SEQ ID NO: 123 - protein, 7 aa, synthetic construct
  REGION 1..7: note = synthetic construct
  SITE 5: note = X is L-2-naphthylalanine
RRFRARQ

SEQ ID NO: 124 - protein, 8 aa, synthetic construct
  REGION 1..8: note = synthetic construct
  SITE 3: note = X is L-2-naphthylalanine
FFARRRRQ

SEQ ID NO: 125 - protein, 8 aa, synthetic construct
  REGION 1..8: note = synthetic construct
  SITE 6: note = X is L-2-naphthylalanine
RFRFRARQ

SEQ ID NO: 126 - protein, 6 aa, synthetic construct
  REGION 1..6: note = synthetic construct
  SITE 2: note = X is L-2-naphthylalanine
FARRRQ

SEQ ID NO: 127 - protein, 7 aa, synthetic construct
  REGION 1..7: note = synthetic construct
  SITE 6: note = X is L-2-naphthylalanine
FRRRRAQ

SEQ ID NO: 128 - protein, 7 aa, synthetic construct
  REGION 1..7: note = synthetic construct
  SITE 1: note = X is D-arginine
  SITE 5: note = X is L-2-naphthylalanine
RRFRARQ

SEQ ID NO: 129 - protein, 7 aa, synthetic construct
  REGION 1..7: note = synthetic construct
  SITE 3: note = X is L-2-naphthylalanine
RRAFRRQ

SEQ ID NO: 130 - protein, 200 aa, synthetic construct
  REGION 1..200: note = synthetic construct
  VARIANT 6..200: note = up to 195 residues may be absent in groups of 5
RRRRRRRRRRRRRRRRRRRRRRRRRRRRRRRRRRRRRRRRRRRRRRRRRRRRRRRRRRRRRRRRRRRRRRRRRRRRRRRRRRRRRRRRRRRRRRRRRRRRRRRRRRRRRRRRRRRRRRRRRRRRRRRRRRRRRRRRRRRRRRRRRRRRRRRRRRRRRRRRRRRRRRRRRRRRRRRRRRRRRRRRRRRRRRRRRRRRRRRR

SEQ ID NO: 131 - protein, 10 aa, synthetic construct
  REGION 1..10: note = synthetic construct
  VARIANT 2..9: note = up to 5 may be absent
CRRRRRRRRC

SEQ ID NO: 132 - protein, 11 aa, synthetic construct
  REGION 1..11: note = synthetic construct
  SITE 2: note = BAla
  VARIANT 3..10: note = up to 5 positions may be absent in this region
  REGION 3..10: note = up to 5 positions may be absent in this region
CARRRRRRRRC

SEQ ID NO: 133 - protein, 11 aa, synthetic construct
  REGION 1..11: note = synthetic construct
  VARIANT 2..9: note = up to 5 positions may be absent in this region
  REGION 2..9: note = up to 5 positions may be absent in this region
  SITE 10: note = bAla
CRRRRRRRRAC

SEQ ID NO: 134 - protein, 12 aa, synthetic construct
  REGION 1..12: note = synthetic construct
  VARIANT 2: note = X can be any naturally occurring amino acid
  VARIANT 11: note = X can be any naturally occurring amino acid
CXRRRRRRRRXC

SEQ ID NO: 135 - protein, 4 aa, synthetic construct
  REGION 1..4: note = synthetic construct
  SITE 2..3: note = bAla
  SITE 3: note = bAla
  SITE 2..3: note = beta-alanine residues are joined by a polyamine of 3 to 8 subunits of which up to 5 may be absent
CAAC

SEQ ID NO: 136 - protein, 7 aa, synthetic construct
  REGION 1..7: note = synthetic construct
CRRRRRC

SEQ ID NO: 137 - RNA, 21 nt, synthetic construct
  modified_base 20..21: mod_base = OTHER; note = thymine
  misc_feature 1..21: note = siLuc siRNA sequence
  source 1..21: mol_type = other RNA
cttacgctgagtacttcgatt

SEQ ID NO: 138 - RNA, 21 nt, synthetic construct
  modified_base 20..21: mod_base = OTHER; note = thymine
  misc_feature 1..21: note = siLuc siRNA sequence
  source 1..21: mol_type = other RNA
tcgaagtactcagcgtaagtt

SEQ ID NO: 139 - DNA, 21 bp, synthetic construct
  misc_feature 1..21: note = DNA/RNA hybrid molecule
  modified_base 3: mod_base = cm
  modified_base 5: mod_base = cm
  modified_base 6: mod_base = um
  modified_base 10: mod_base = cm
  modified_base 12..13: mod_base = um
  modified_base 16: mod_base = um
  modified_base 17: mod_base = cm
  misc_feature 1..19: note = RNA
  misc_feature 20..21: note = DNA
  source 1..21: mol_type = other DNA
aacgctgggcgttaatcaatt

SEQ ID NO: 140 - DNA, 21 bp, synthetic construct
  misc_feature 1..21: note = DNA/RNA hybrid molecule
  modified_base 6: mod_base = um
  modified_base 13: mod_base = cm
  misc_feature 1..19: note = RNA
  misc_feature 20..21: note = DNA
  source 1..21: mol_type = other DNA
ttgattaacgcccagcgtttt

SEQ ID NO: 141 - protein, 8 aa, synthetic construct
  REGION 1..8: note = synthetic peptide
  SITE 1: note = X is D-phenylalanine
  SITE 2: note = X is L-2-naphthylalanine
  SITE 4: note = X is D-arginine
  SITE 6: note = X is D-arginine
  MOD_RES 7..8: note = Gln and Cys are joined by a miniPEG (diethylene glycol) moiety
FARRRRQC

SEQ ID NO: 142 - protein, 5 aa, synthetic construct
  REGION 1..5: note = synthetic construct
RRRRR

SEQ ID NO: 143 - protein, 6 aa, synthetic construct
  REGION 1..6: note = synthetic construct
RRRRRR

SEQ ID NO: 144 - protein, 20 aa, synthetic construct
  REGION 1..20: note = synthetic construct
RRRRRSSRRRRRRSSRRRRR

SEQ ID NO: 145 - protein, 6 aa, synthetic construct
  REGION 1..6: note = synthetic construct
RRRRRC